European Patent Application EP 4 741 012 A2, published May 13, 2026. Title: COMPOSITIONS AND METHODS FOR REDUCING AMYLOID BETA FORMATION AND COMPOSITION THEREFORE. Applicant: ARIBIO CO., LTD. Application EP 26152136.3, filed March 24, 2020. The sequence listing filed with the application follows.

SEQUENCE LISTING (18 sequences)

SEQ ID NO: 1 - DNA, 20 bp, synthetic construct
  source 1..20: mol_type = other DNA
ctggtatacacccatccggc

SEQ ID NO: 2 - DNA, 20 bp, synthetic construct
  source 1..20: mol_type = other DNA
cttgggcaaacgaaggttgg

SEQ ID NO: 3 - DNA, 18 bp, synthetic construct
  source 1..18: mol_type = other DNA
ccaggtcatcaccattgg

SEQ ID NO: 4 - DNA, 18 bp, synthetic construct
  source 1..18: mol_type = other DNA
cagagtacttgcgctcag

SEQ ID NO: 5 - DNA, 21 bp, synthetic construct
  source 1..21: mol_type = other DNA
attccaacgctatcaagaacc

SEQ ID NO: 6 - DNA, 22 bp, synthetic construct
  source 1..22: mol_type = other DNA
ccaaggtgctatgatcattacc

SEQ ID NO: 7 - DNA, 19 bp, synthetic construct
  source 1..19: mol_type = other DNA
tctgctaggagccagtgcc

SEQ ID NO: 8 - DNA, 21 bp, synthetic construct
  source 1..21: mol_type = other DNA
gatggtgatctttctgtatcc

SEQ ID NO: 9 - DNA, 19 bp, synthetic construct
  source 1..19: mol_type = other DNA
ctgtccctgtatgcctctg

SEQ ID NO: 10 - DNA, 18 bp, synthetic construct
  source 1..18: mol_type = other DNA
atgtcacgcacgatttcc

SEQ ID NO: 11 - DNA, 22 bp, synthetic construct
  source 1..22: mol_type = other DNA
ctctttggccgagagttcgtgg

SEQ ID NO: 12 - DNA, 22 bp, synthetic construct
  source 1..22: mol_type = other DNA
cctcggttgccgtaaaggacgc

SEQ ID NO: 13 - DNA, 22 bp, synthetic construct
  source 1..22: mol_type = other DNA
ctcgcatggcatagatgggtgc

SEQ ID NO: 14 - DNA, 21 bp, synthetic construct
  source 1..21: mol_type = other DNA
gcaggtgtgcacgtcatagac

SEQ ID NO: 15 - DNA, 20 bp, synthetic construct
  source 1..20: mol_type = other DNA
catggagtgtctggctcctg

SEQ ID NO: 16 - DNA, 22 bp, synthetic construct
  source 1..22: mol_type = other DNA
gtccatcccctctgaggtcttg

SEQ ID NO: 17 - DNA, 20 bp, synthetic construct
  source 1..20: mol_type = other DNA
cgggagatcaagcagaatgc

SEQ ID NO: 18 - DNA, 22 bp, synthetic construct
  source 1..22: mol_type = other DNA
gcctagctctcggaactgtggc